European Patent Application EP 4 807 003 A1, published September 16, 2026. Title: METHOD AND COMPOUNDS TO ADDRESS AGEING. Applicant: Resalis therapeutics s.r.l. The sequence listing filed with the application follows.

SEQUENCE LISTING (20 sequences)

SEQ ID NO: 1 - RNA, 22 nt, Homo sapiens
  source 1..22: mol_type = other RNA
aagctgccagttgaagaactgt

SEQ ID NO: 2 - skipped

SEQ ID NO: 3 - DNA, 15 bp, synthetic construct
  misc_feature 1..15: note = Synthetic Nucleic Acid
  source 1..15: mol_type = other DNA
cttcaactggcagct

SEQ ID NO: 4 - DNA, 16 bp, synthetic construct
  misc_feature 1..16: note = Synthetic Nucleic Acid
  source 1..16: mol_type = other DNA
tcttcaactggcagct

SEQ ID NO: 5 - DNA, 17 bp, synthetic construct
  misc_feature 1..17: note = Synthetic Nucleic Acid
  source 1..17: mol_type = other DNA
ttcttcaactggcagct

SEQ ID NO: 6 - DNA, 18 bp, synthetic construct
  misc_feature 1..18: note = Synthetic Nucleic Acid
  source 1..18: mol_type = other DNA
gttcttcaactggcagct

SEQ ID NO: 7 - DNA, 15 bp, synthetic construct
  misc_feature 1..15: note = Synthetic Nucleic Acid
  source 1..15: mol_type = other DNA
cttcaactggcagct

SEQ ID NO: 8 - DNA, 15 bp, synthetic construct
  misc_feature 1..15: note = Synthetic Nucleic Acid
  source 1..15: mol_type = other DNA
cttcaactggcagct

SEQ ID NO: 9 - DNA, 16 bp, synthetic construct
  misc_feature 1..16: note = Synthetic Nucleic Acid
  source 1..16: mol_type = other DNA
tcttcaactggcagct

SEQ ID NO: 10 - DNA, 16 bp, synthetic construct
  misc_feature 1..16: note = Synthetic Nucleic Acid
  source 1..16: mol_type = other DNA
tcttcaactggcagct

SEQ ID NO: 11 - DNA, 16 bp, synthetic construct
  misc_feature 1..16: note = Synthetic Nucleic Acid
  source 1..16: mol_type = other DNA
tcttcaactggcagct

SEQ ID NO: 12 - DNA, 17 bp, synthetic construct
  misc_feature 1..17: note = Synthetic Nucleic Acid
  source 1..17: mol_type = other DNA
ttcttcaactggcagct

SEQ ID NO: 13 - DNA, 18 bp, synthetic construct
  misc_feature 1..18: note = Synthetic Nucleic Acid
  source 1..18: mol_type = other DNA
gttcttcaactggcagct

SEQ ID NO: 14 - DNA, 16 bp, synthetic construct
  misc_feature 1..16: note = Synthetic Nucleic Acid
  source 1..16: mol_type = other DNA
cgaatagttagtagcg

SEQ ID NO: 15 - DNA, 16 bp, synthetic construct
  misc_feature 1..16: note = Synthetic Nucleic Acid
  source 1..16: mol_type = other DNA
cgaatagttagtagcg

SEQ ID NO: 16 - DNA, 18 bp, synthetic construct
  source 1..18: mol_type = other DNA
gttcttcaactggcagct

SEQ ID NO: 17 - DNA, 18 bp, synthetic construct
  source 1..18: mol_type = other DNA
gttcttcaactggcagct

SEQ ID NO: 18 - DNA, 18 bp, synthetic construct
  source 1..18: mol_type = other DNA
gttcttcaactggcagct

SEQ ID NO: 19 - DNA, 18 bp, synthetic construct
  source 1..18: mol_type = other DNA
gttcttcaactggcagct

SEQ ID NO: 20 - DNA, 18 bp, synthetic construct
  source 1..18: mol_type = other DNA
gttcttcaactggcagct